European Patent Specification EP 3 823 664 B1, published January 8, 2025. Title: Bispecific Anti-BCMA X Anti-CD3 Antibodies and Uses Thereof. Applicant: Regeneron Pharmaceuticals, Inc. The sequence listing filed with the application follows.

SEQUENCE LISTING (125 sequences)

SEQ ID NO: 1 - DNA, 366 bp, Artificial Sequence
  synthetic
caggtgcagctggtggagtcggggggaggcgtggtccagcctgggaggtccctgagactctcctgtgcagcctctggattcaccttcagtacctatggcattcactgggtccgccaggctccaggcaaggggctggagtgggtggcagttatattacatgatggaagtagtaactactatgcagagtccgtgaagggccgattcatcatctccagagacaattccaagaacacactgtatctgcaaatgaacagcctgagagctgaggacacggctctatattactgtacgaaaaggtattcagaagcagctggcccaaattggttcgacccctggggccagggaaccctggtcaccgtctcctca

SEQ ID NO: 2 - protein, 122 aa, Artificial Sequence
  synthetic
QVQLVESGGGVVQPGRSLRLSCAASGFTFSTYGIHWVRQAPGKGLEWVAVILHDGSSNYYAESVKGRFIISRDNSKNTLYLQMNSLRAEDTALYYCTKRYSEAAGPNWFDPWGQGTLVTVSS

SEQ ID NO: 3 - DNA, 24 bp, Artificial Sequence
  synthetic
ggattcaccttcagtacctatggc

SEQ ID NO: 4 - protein, 8 aa, Artificial Sequence
  synthetic
GFTFSTYG

SEQ ID NO: 5 - DNA, 24 bp, Artificial Sequence
  synthetic
atattacatgatggaagtagtaac

SEQ ID NO: 6 - protein, 8 aa, Artificial Sequence
  synthetic
ILHDGSSN

SEQ ID NO: 7 - DNA, 45 bp, Artificial Sequence
  synthetic
acgaaaaggtattcagaagcagctggcccaaattggttcgacccc

SEQ ID NO: 8 - protein, 15 aa, Artificial Sequence
  synthetic
TKRYSEAAGPNWFDP

SEQ ID NO: 9 - DNA, 321 bp, Artificial Sequence
  synthetic
gacatccagatgacccagtctccatcctccgtgtctgcatctgtaggagacagagtcaccatcacttgtcgggcgagtcggggaattagcagctggttagcctggtatcagcagaagccagggaaagcccctaagctcctgatccatgctgcatccagtttgcaaagtggggtcccatcaaggttcagcggcagtggatctgggacagatttcactctcaccatcagcagcctgcagcctgaagattttgctacttactattgtcaacaggctatcagtttcccattcactttcggccctgggaccaaagtggatatcaaa

SEQ ID NO: 10 - protein, 107 aa, Artificial Sequence
  synthetic
DIQMTQSPSSVSASVGDRVTITCRASRGISSWLAWYQQKPGKAPKLLIHAASSLQSGVPSRFSGSGSGTDFTLTISSLQPEDFATYYCQQAISFPFTFGPGTKVDIK

SEQ ID NO: 11 - DNA, 18 bp, Artificial Sequence
  synthetic
cggggaattagcagctgg

SEQ ID NO: 12 - protein, 6 aa, Artificial Sequence
  synthetic
RGISSW

SEQ ID NO: 13 - DNA, 9 bp, Artificial Sequence
  synthetic
gctgcatcc

SEQ ID NO: 14 - protein, 3 aa, Artificial Sequence
  synthetic
AAS

SEQ ID NO: 15 - DNA, 27 bp, Artificial Sequence
  synthetic
caacaggctatcagtttcccattcact

SEQ ID NO: 16 - protein, 9 aa, Artificial Sequence
  synthetic
QQAISFPFT

SEQ ID NO: 17 - DNA, 360 bp, Artificial Sequence
  synthetic
gaggtgcagctggtggagtctgggggaggcttggtacagcctggggggtccctgagactctcctgtgcagcctctggattcacctttagcagctatgtcatgagttgggtccgccaggctccagggaagggactggagtgggtctcagctattattggtagtggtggtagcacatattacgcagactccgtgaagggccggttcaccatctccagagacaattccaagaacacgctgtatctgcaaatgaacagcctgagagccgaggacacggccgtatattactgtgcgaaaagagccggggataactggaactggttcgacccctggggccagggaaccctggtcaccgtctcctca

SEQ ID NO: 18 - protein, 120 aa, Artificial Sequence
  synthetic
EVQLVESGGGLVQPGGSLRLSCAASGFTFSSYVMSWVRQAPGKGLEWVSAIIGSGGSTYYADSVKGRFTISRDNSKNTLYLQMNSLRAEDTAVYYCAKRAGDNWNWFDPWGQGTLVTVSS

SEQ ID NO: 19 - DNA, 24 bp, Artificial Sequence
  synthetic
ggattcacctttagcagctatgtc

SEQ ID NO: 20 - protein, 8 aa, Artificial Sequence
  synthetic
GFTFSSYV

SEQ ID NO: 21 - DNA, 24 bp, Artificial Sequence
  synthetic
attattggtagtggtggtagcaca

SEQ ID NO: 22 - protein, 8 aa, Artificial Sequence
  synthetic
IIGSGGST

SEQ ID NO: 23 - DNA, 39 bp, Artificial Sequence
  synthetic
gcgaaaagagccggggataactggaactggttcgacccc

SEQ ID NO: 24 - protein, 13 aa, Artificial Sequence
  synthetic
AKRAGDNWNWFDP

SEQ ID NO: 25 - DNA, 321 bp, Artificial Sequence
  synthetic
gacatccagatgacccagtctccatcttccgtgtctgcatctttaggagacagagtcaccatcacttgtcgggcgagtcagggtattagcagctggttagcctggtatcagcggaaaccagggaaagcccctaagctcctgatctatgctgcatccagtttgcaaagtggggtcccatcaaggttcagcggcagtggatctggggcggatttcactctcaccatcagcagcctgcagcctgaagattttgcaacttactattgtcaacaggctaaaagtgtcccattcactttcggccctgggaccaaagtggatatcaaa

SEQ ID NO: 26 - protein, 107 aa, Artificial Sequence
  synthetic
DIQMTQSPSSVSASLGDRVTITCRASQGISSWLAWYQRKPGKAPKLLIYAASSLQSGVPSRFSGSGSGADFTLTISSLQPEDFATYYCQQAKSVPFTFGPGTKVDIK

SEQ ID NO: 27 - DNA, 18 bp, Artificial Sequence
  synthetic
cagggtattagcagctgg

SEQ ID NO: 28 - protein, 6 aa, Artificial Sequence
  synthetic
QGISSW

SEQ ID NO: 29 - DNA, 9 bp, Artificial Sequence
  synthetic
gctgcatcc

SEQ ID NO: 30 - protein, 3 aa, Artificial Sequence
  synthetic
AAS

SEQ ID NO: 31 - DNA, 27 bp, Artificial Sequence
  synthetic
caacaggctaaaagtgtcccattcact

SEQ ID NO: 32 - protein, 9 aa, Artificial Sequence
  synthetic
QQAKSVPFT

SEQ ID NO: 33 - DNA, 351 bp, Artificial Sequence
  synthetic
gaagtgcagctggtggagtctgggggaggcttggtacagcctggcaggtccctgagactctcctgtgcagcctctggattcacctttgatgattatgccatgcactgggtccggcaagctccagggaagggcctggagtgggtctcaggtatcagttggaatagtggtaacatgggatatgcggactctgtgaagggccgattcaccatctccagagacaacgccaagaactccctgttcctgcaaatgcacagtttgagagctgaggacacggccttttattactgtgcaaaagtccgtctaactgcctttgacttttggggccagggaaccctggtcaccgtctcctca

SEQ ID NO: 34 - protein, 117 aa, Artificial Sequence
  synthetic
EVQLVESGGGLVQPGRSLRLSCAASGFTFDDYAMHWVRQAPGKGLEWVSGISWNSGNMGYADSVKGRFTISRDNAKNSLFLQMHSLRAEDTAFYYCAKVRLTAFDFWGQGTLVTVSS

SEQ ID NO: 35 - DNA, 24 bp, Artificial Sequence
  synthetic
ggattcacctttgatgattatgcc

SEQ ID NO: 36 - protein, 8 aa, Artificial Sequence
  synthetic
GFTFDDYA

SEQ ID NO: 37 - DNA, 24 bp, Artificial Sequence
  synthetic
atcagttggaatagtggtaacatg

SEQ ID NO: 38 - protein, 8 aa, Artificial Sequence
  synthetic
ISWNSGNM

SEQ ID NO: 39 - DNA, 30 bp, Artificial Sequence
  synthetic
gcaaaagtccgtctaactgcctttgacttt

SEQ ID NO: 40 - protein, 10 aa, Artificial Sequence
  synthetic
AKVRLTAFDF

SEQ ID NO: 41 - DNA, 321 bp, Artificial Sequence
  synthetic
gacatccagatgacccagtctccatcctccctgtctgcatctgtaggagacagagtcaccatcacttgccggacaagtcagagcattggcaactatttaaattggtttcagcagaaaccagggaaagcccctaaactcctcatctatactgcatccagtttgcagaatggagtcccatcaaggttcactggcagtggatctgggacagatttcactctcaccatcagcagtctgcaacctgaggattttgtaatttactactgtcaacagagtttcagtaccccgtatacttttggccaggggaccaagctggagatcaaa

SEQ ID NO: 42 - protein, 107 aa, Artificial Sequence
  synthetic
DIQMTQSPSSLSASVGDRVTITCRTSQSIGNYLNWFQQKPGKAPKLLIYTASSLQNGVPSRFTGSGSGTDFTLTISSLQPEDFVIYYCQQSFSTPYTFGQGTKLEIK

SEQ ID NO: 43 - DNA, 18 bp, Artificial Sequence
  synthetic
cagagcattggcaactat

SEQ ID NO: 44 - protein, 6 aa, Artificial Sequence
  synthetic
QSIGNY

SEQ ID NO: 45 - DNA, 9 bp, Artificial Sequence
  synthetic
actgcatcc

SEQ ID NO: 46 - protein, 3 aa, Artificial Sequence
  synthetic
TAS

SEQ ID NO: 47 - DNA, 27 bp, Artificial Sequence
  synthetic
caacagagtttcagtaccccgtatact

SEQ ID NO: 48 - protein, 9 aa, Artificial Sequence
  synthetic
QQSFSTPYT

SEQ ID NO: 49 - DNA, 354 bp, Artificial Sequence
  synthetic
caggtgcagctggtggagtctgggggaggcttggtcaagcctggagggtccctgagactctcctgtgcagcctctggattcaccttcagtgactactacatcagctggatccgccaggctccagggaaggggctggagtgggtttcatacattagttctagtggtagttccataaagtacgcagactctgtgaagggccgattcaccatctccagggacaacgccaagaactcactgtatctgcaaatgaacagcctgagagccgaggacacggccgtatattactgtgcgagagagggagggaactacggtatggacgtctggggccaagggaccacggtcaccgtctcctca

SEQ ID NO: 50 - protein, 118 aa, Artificial Sequence
  synthetic
QVQLVESGGGLVKPGGSLRLSCAASGFTFSDYYISWIRQAPGKGLEWVSYISSSGSSIKYADSVKGRFTISRDNAKNSLYLQMNSLRAEDTAVYYCAREGGNYGMDVWGQGTTVTVSS

SEQ ID NO: 51 - DNA, 24 bp, Artificial Sequence
  synthetic
ggattcaccttcagtgactactac

SEQ ID NO: 52 - protein, 8 aa, Artificial Sequence
  synthetic
GFTFSDYY

SEQ ID NO: 53 - DNA, 24 bp, Artificial Sequence
  synthetic
attagttctagtggtagttccata

SEQ ID NO: 54 - protein, 8 aa, Artificial Sequence
  synthetic
ISSSGSSI

SEQ ID NO: 55 - DNA, 33 bp, Artificial Sequence
  synthetic
gcgagagagggagggaactacggtatggacgtc

SEQ ID NO: 56 - protein, 11 aa, Artificial Sequence
  synthetic
AREGGNYGMDV

SEQ ID NO: 57 - DNA, 321 bp, Artificial Sequence
  synthetic
gacatccagatgacccagtctccatcttccgtgtctgcatctgtaggagacagagtcaccatcacttgtcgggcgagtcagggtattaacaactggttagtctggtatcagcagaaaccagggaaagcccctaagctcctgatctatgctgcaaccagcttgcaaagtggggtcccatcaaggttcagcggcagtgggtctgggacagatttcactctcaccatcagcagcctgcagcctgaagattttgcaacttactattgtcaacaggctaacagtttccctcccacttttggccaggggaccaagctggagatcaaa

SEQ ID NO: 58 - protein, 107 aa, Artificial Sequence
  synthetic
DIQMTQSPSSVSASVGDRVTITCRASQGINNWLVWYQQKPGKAPKLLIYAATSLQSGVPSRFSGSGSGTDFTLTISSLQPEDFATYYCQQANSFPPTFGQGTKLEIK

SEQ ID NO: 59 - DNA, 18 bp, Artificial Sequence
  synthetic
cagggtattaacaactgg

SEQ ID NO: 60 - protein, 6 aa, Artificial Sequence
  synthetic
QGINNW

SEQ ID NO: 61 - DNA, 9 bp, Artificial Sequence
  synthetic
gctgcaacc

SEQ ID NO: 62 - protein, 3 aa, Artificial Sequence
  synthetic
AAT

SEQ ID NO: 63 - DNA, 27 bp, Artificial Sequence
  synthetic
caacaggctaacagtttccctcccact

SEQ ID NO: 64 - protein, 9 aa, Artificial Sequence
  synthetic
QQANSFPPT

SEQ ID NO: 65 - DNA, 375 bp, Artificial Sequence
  synthetic
gaggtgcagctggtggagtctgggggaggcttggtccagcctggggggtccctgagactctcctgtgcagcctctggattcacctttagtaacttttggatgacctgggtccgccaggctccagggaaggggctggagtgggtggccaacatgaaccaagatggaagtgagaaatactatgtggactctgtgaagggccgattcaccatctccagagacaacgccaagagctcactgtatctgcaaatgaacagcctgagagccgaggacacggctgtgtattactgtgcgagagatcgggaatattgtattagtaccagctgctatgatgactttgactactggggccagggaaccctggtcaccgtctcctca

SEQ ID NO: 66 - protein, 125 aa, Artificial Sequence
  synthetic
EVQLVESGGGLVQPGGSLRLSCAASGFTFSNFWMTWVRQAPGKGLEWVANMNQDGSEKYYVDSVKGRFTISRDNAKSSLYLQMNSLRAEDTAVYYCARDREYCISTSCYDDFDYWGQGTLVTVSS

SEQ ID NO: 67 - DNA, 24 bp, Artificial Sequence
  synthetic
ggattcacctttagtaacttttgg

SEQ ID NO: 68 - protein, 8 aa, Artificial Sequence
  synthetic
GFTFSNFW

SEQ ID NO: 69 - DNA, 24 bp, Artificial Sequence
  synthetic
atgaaccaagatggaagtgagaaa

SEQ ID NO: 70 - protein, 8 aa, Artificial Sequence
  synthetic
MNQDGSEK

SEQ ID NO: 71 - DNA, 54 bp, Artificial Sequence
  synthetic
gcgagagatcgggaatattgtattagtaccagctgctatgatgactttgactac

SEQ ID NO: 72 - protein, 18 aa, Artificial Sequence
  synthetic
ARDREYCISTSCYDDFDY

SEQ ID NO: 73 - DNA, 324 bp, Artificial Sequence
  synthetic
gacatccagatgacccagtctccatcctccctgtctgcatctgtaggagacagagtcaccatcacttgccgggcaagtcagagcattagcagctatttaaattggtatcagcagaaaccagggaaagcccctaagctcctgatctatgctgcatccagtttgcatagtggggtcccatcaaggttcagtggcagtggatctgggacagatttcactctcaccatcagcagtctgcaacctgaagattttgcaacttactactgtcaacagagttacagtacccctccgatcaccttcggccaagggacacgactggagattaaa

SEQ ID NO: 74 - protein, 108 aa, Artificial Sequence
  synthetic
DIQMTQSPSSLSASVGDRVTITCRASQSISSYLNWYQQKPGKAPKLLIYAASSLHSGVPSRFSGSGSGTDFTLTISSLQPEDFATYYCQQSYSTPPITFGQGTRLEIK

SEQ ID NO: 75 - DNA, 18 bp, Artificial Sequence
  synthetic
cagagcattagcagctat

SEQ ID NO: 76 - protein, 6 aa, Artificial Sequence
  synthetic
QSISSY

SEQ ID NO: 77 - DNA, 9 bp, Artificial Sequence
  synthetic
gctgcatcc

SEQ ID NO: 78 - protein, 3 aa, Artificial Sequence
  synthetic
AAS

SEQ ID NO: 79 - DNA, 30 bp, Artificial Sequence
  synthetic
caacagagttacagtacccctccgatcacc

SEQ ID NO: 80 - protein, 10 aa, Artificial Sequence
  synthetic
QQSYSTPPIT

SEQ ID NO: 81 - DNA, 324 bp, Artificial Sequence
  synthetic
gacatccagatgacccagtctccatcctccctgtctgcatctgtaggagacagagtcaccatcacttgccgggcaagtcagagcattagcagctatttaaattggtatcagcagaaaccagggaaagcccctaagctcctgatctatgctgcatccagtttgcaaagtggggtcccgtcaaggttcagtggcagtggatctgggacagatttcactctcaccatcagcagtctgcaacctgaagattttgcaacttactactgtcaacagagttacagtacccctccgatcaccttcggccaagggacacgactggagattaaa

SEQ ID NO: 82 - protein, 108 aa, Artificial Sequence
  synthetic
DIQMTQSPSSLSASVGDRVTITCRASQSISSYLNWYQQKPGKAPKLLIYAASSLQSGVPSRFSGSGSGTDFTLTISSLQPEDFATYYCQQSYSTPPITFGQGTRLEIK

SEQ ID NO: 83 - DNA, 18 bp, Artificial Sequence
  synthetic
cagagcattagcagctat

SEQ ID NO: 84 - protein, 6 aa, Artificial Sequence
  synthetic
QSISSY

SEQ ID NO: 85 - DNA, 9 bp, Artificial Sequence
  synthetic
gctgcatcc

SEQ ID NO: 86 - protein, 3 aa, Artificial Sequence
  synthetic
AAS

SEQ ID NO: 87 - DNA, 30 bp, Artificial Sequence; identical to SEQ ID NO: 79
  synthetic

SEQ ID NO: 88 - protein, 10 aa, Artificial Sequence
  synthetic
QQSYSTPPIT

SEQ ID NO: 89 - DNA, 372 bp, Artificial Sequence
  synthetic
gaagtacagcttgtagaatccggcggaggactggtacaacctggaagaagtcttagactgagttgcgcagctagtgggtttacattcgacgattacagcatgcattgggtgaggcaagctcctggtaaaggattggaatgggttagcgggatatcatggaactcaggaagcaagggatacgccgacagcgtgaaaggccgatttacaatatctagggacaacgcaaaaaactctctctaccttcaaatgaactctcttagggcagaagacacagcattgtattattgcgcaaaatacggcagtggttatggcaagttttatcattatggactggacgtgtggggacaagggacaacagtgacagtgagtagc

SEQ ID NO: 90 - protein, 124 aa, Artificial Sequence
  synthetic
EVQLVESGGGLVQPGRSLRLSCAASGFTFDDYSMHWVRQAPGKGLEWVSGISWNSGSKGYADSVKGRFTISRDNAKNSLYLQMNSLRAEDTALYYCAKYGSGYGKFYHYGLDVWGQGTTVTVSS

SEQ ID NO: 91 - DNA, 24 bp, Artificial Sequence
  synthetic
gggtttacattcgacgattacagc

SEQ ID NO: 92 - protein, 8 aa, Artificial Sequence
  synthetic
GFTFDDYS

SEQ ID NO: 93 - DNA, 24 bp, Artificial Sequence
  synthetic
atatcatggaactcaggaagcaag

SEQ ID NO: 94 - protein, 8 aa, Artificial Sequence
  synthetic
ISWNSGSK

SEQ ID NO: 95 - DNA, 51 bp, Artificial Sequence
  synthetic
gcaaaatacggcagtggttatggcaagttttatcattatggactggacgtg

SEQ ID NO: 96 - protein, 17 aa, Artificial Sequence
  synthetic
AKYGSGYGKFYHYGLDV

SEQ ID NO: 97 - DNA, 372 bp, Artificial Sequence
  synthetic
gaagtacagcttgtagaatccggcggaggactggtacaacctggaagaagtcttagactgagttgcgcagctagtgggtttacattcgacgattacagcatgcattgggtgaggcaagctcctggtaaaggattggaatgggttagcgggatatcatggaactcaggaagcatcggatacgccgacagcgtgaaaggccgatttacaatatctagggacaacgcaaaaaactctctctaccttcaaatgaactctcttagggcagaagacacagcattgtattattgcgcaaaatacggcagtggttatggcaagttttattattatggaatggacgtgtggggacaagggacaacagtgacagtgagtagc

SEQ ID NO: 98 - protein, 124 aa, Artificial Sequence
  synthetic
EVQLVESGGGLVQPGRSLRLSCAASGFTFDDYSMHWVRQAPGKGLEWVSGISWNSGSIGYADSVKGRFTISRDNAKNSLYLQMNSLRAEDTALYYCAKYGSGYGKFYYYGMDVWGQGTTVTVSS

SEQ ID NO: 99 - DNA, 24 bp, Artificial Sequence
  synthetic
gggtttacattcgacgattacagc

SEQ ID NO: 100 - protein, 8 aa, Artificial Sequence
  synthetic
GFTFDDYS

SEQ ID NO: 101 - DNA, 24 bp, Artificial Sequence
  synthetic
atatcatggaactcaggaagcatc

SEQ ID NO: 102 - protein, 8 aa, Artificial Sequence
  synthetic
ISWNSGSI

SEQ ID NO: 103 - DNA, 51 bp, Artificial Sequence
  synthetic
gcaaaatacggcagtggttatggcaagttttattattatggaatggacgtg

SEQ ID NO: 104 - protein, 17 aa, Artificial Sequence
  synthetic
AKYGSGYGKFYYYGMDV

SEQ ID NO: 105 - DNA, 249 bp, Artificial Sequence
  hBCMA ecto.mmh
atgttgcagatggctgggcagtgctcccaaaatgaatattttgacagtttgttgcatgcttgcataccttgtcaacttcgatgttcttctaatactcctcctctaacatgtcagcgttattgtaatgcaagtgtgaccaattcagtgaaaggaacgaatgcggaacaaaaactcatctcagaagaggatctgggtggagaacaaaaactcatctcagaagaggatctgcaccatcaccatcaccattga

SEQ ID NO: 106 - protein, 82 aa, Artificial Sequence
  hBCMA ecto.mmh
MLQMAGQCSQNEYFDSLLHACIPCQLRCSSNTPPLTCQRYCNASVTNSVKGTNAEQKLISEEDLGGEQKLISEEDLHHHHHH

SEQ ID NO: 107 - DNA, 864 bp, Artificial Sequence
  hBCMA ecto.mFc
atgttgcagatggctgggcagtgctcccaaaatgaatattttgacagtttgttgcatgcttgcataccttgtcaacttcgatgttcttctaatactcctcctctaacatgtcagcgttattgtaatgcaagtgtgaccaattcagtgaaaggaacgaatgcggagcccagagggcccacaatcaagccctgtcctccatgcaaatgcccagcacctaacctcttgggtggaccatccgtcttcatcttccctccaaagatcaaggatgtactcatgatctccctgagccccatagtcacatgtgtggtggtggatgtgagcgaggatgacccagatgtccagatcagctggtttgtgaacaacgtggaagtacacacagctcagacacaaacccatagagaggattacaacagtactctccgggtggtcagtgccctccccatccagcaccaggactggatgagtggcaaggagttcaaatgcaaggtcaacaacaaagacctcccagcgcccatcgagagaaccatctcaaaacccaaagggtcagtaagagctccacaggtatatgtcttgcctccaccagaagaagagatgactaagaaacaggtcactctgacctgcatggtcacagacttcatgcctgaagacatttacgtggagtggaccaacaacgggaaaacagagctaaactacaagaacactgaaccagtcctggactctgatggttcttacttcatgtacagcaagctgagagtggaaaagaagaactgggtggaaagaaatagctactcctgttcagtggtccacgagggtctgcacaatcaccacacgactaagagcttctcccggactccgggtaaatga

SEQ ID NO: 108 - protein, 287 aa, Artificial Sequence
  hBCMA ecto.mFc
MLQMAGQCSQNEYFDSLLHACIPCQLRCSSNTPPLTCQRYCNASVTNSVKGTNAEPRGPTIKPCPPCKCPAPNLLGGPSVFIFPPKIKDVLMISLSPIVTCVVVDVSEDDPDVQISWFVNNVEVHTAQTQTHREDYNSTLRVVSALPIQHQDWMSGKEFKCKVNNKDLPAPIERTISKPKGSVRAPQVYVLPPPEEEMTKKQVTLTCMVTDFMPEDIYVEWTNNGKTELNYKNTEPVLDSDGSYFMYSKLRVEKKNWVERNSYSCSVVHEGLHNHHTTKSFSRTPGK

SEQ ID NO: 109 - DNA, 246 bp, Artificial Sequence
  mfBCMA ecto.mmh
atgttgcagatggctcggcagtgctcccaaaatgaatattttgacagtttgttgcatgattgcaaaccttgtcaacttcgatgttctagtactcctcctctaacatgtcagcgttattgcaatgcaagtatgaccaattcagtgaaaggaatgaatgcggaacaaaaactcatctcagaagaggatctgggtggagaacaaaaactcatctcagaagaggatctgcaccatcaccatcaccattga

SEQ ID NO: 110 - protein, 81 aa, Artificial Sequence
  mfBCMA ecto.mmh
MLQMARQCSQNEYFDSLLHDCKPCQLRCSSTPPLTCQRYCNASMTNSVKGMNAEQKLISEEDLGGEQKLISEEDLHHHHHH

SEQ ID NO: 111 - DNA, 861 bp, Artificial Sequence
  mfBCMA ecto.mFc
atgttgcagatggctcggcagtgctcccaaaatgaatattttgacagtttgttgcatgattgcaaaccttgtcaacttcgatgttctagtactcctcctctaacatgtcagcgttattgcaatgcaagtatgaccaattcagtgaaaggaatgaatgcggagcccagagggcccacaatcaagccctgtcctccatgcaaatgcccagcacctaacctcttgggtggaccatccgtcttcatcttccctccaaagatcaaggatgtactcatgatctccctgagccccatagtcacatgtgtggtggtggatgtgagcgaggatgacccagatgtccagatcagctggtttgtgaacaacgtggaagtacacacagctcagacacaaacccatagagaggattacaacagtactctccgggtggtcagtgccctccccatccagcaccaggactggatgagtggcaaggagttcaaatgcaaggtcaacaacaaagacctcccagcgcccatcgagagaaccatctcaaaacccaaagggtcagtaagagctccacaggtatatgtcttgcctccaccagaagaagagatgactaagaaacaggtcactctgacctgcatggtcacagacttcatgcctgaagacatttacgtggagtggaccaacaacgggaaaacagagctaaactacaagaacactgaaccagtcctggactctgatggttcttacttcatgtacagcaagctgagagtggaaaagaagaactgggtggaaagaaatagctactcctgttcagtggtccacgagggtctgcacaatcaccacacgactaagagcttctcccggactccgggtaaatga

SEQ ID NO: 112 - protein, 286 aa, Artificial Sequence
  mfBCMA ecto.mFc
MLQMARQCSQNEYFDSLLHDCKPCQLRCSSTPPLTCQRYCNASMTNSVKGMNAEPRGPTIKPCPPCKCPAPNLLGGPSVFIFPPKIKDVLMISLSPIVTCVVVDVSEDDPDVQISWFVNNVEVHTAQTQTHREDYNSTLRVVSALPIQHQDWMSGKEFKCKVNNKDLPAPIERTISKPKGSVRAPQVYVLPPPEEEMTKKQVTLTCMVTDFMPEDIYVEWTNNGKTELNYKNTEPVLDSDGSYFMYSKLRVEKKNWVERNSYSCSVVHEGLHNHHTTKSFSRTPGK

SEQ ID NO: 113 - DNA, 849 bp, Artificial Sequence
  Mouse BCMA ecto domain with mouse Fc
atggcgcaacagtgtttccacagtgaatattttgacagtctgctgcatgcttgcaaaccgtgtcacttgcgatgttccaaccctcctgcaacctgtcagccttactgtgatccaagcgtgaccagttcagtgaaagggacgtacacggagcccagagggcccacaatcaagccctgtcctccatgcaaatgcccagcacctaacctcttgggtggaccatccgtcttcatcttccctccaaagatcaaggatgtactcatgatctccctgagccccatagtcacatgtgtggtggtggatgtgagcgaggatgacccagatgtccagatcagctggtttgtgaacaacgtggaagtacacacagctcagacacaaacccatagagaggattacaacagtactctccgggtggtcagtgccctccccatccagcaccaggactggatgagtggcaaggagttcaaatgcaaggtcaacaacaaagacctcccagcgcccatcgagagaaccatctcaaaacccaaagggtcagtaagagctccacaggtatatgtcttgcctccaccagaagaagagatgactaagaaacaggtcactctgacctgcatggtcacagacttcatgcctgaagacatttacgtggagtggaccaacaacgggaaaacagagctaaactacaagaacactgaaccagtcctggactctgatggttcttacttcatgtacagcaagctgagagtggaaaagaagaactgggtggaaagaaatagctactcctgttcagtggtccacgagggtctgcacaatcaccacacgactaagagcttctcccggactccgggtaaatga

SEQ ID NO: 114 - protein, 282 aa, Artificial Sequence
  Mouse BCMA ecto domain with mouse Fc
MAQQCFHSEYFDSLLHACKPCHLRCSNPPATCQPYCDPSVTSSVKGTYTEPRGPTIKPCPPCKCPAPNLLGGPSVFIFPPKIKDVLMISLSPIVTCVVVDVSEDDPDVQISWFVNNVEVHTAQTQTHREDYNSTLRVVSALPIQHQDWMSGKEFKCKVNNKDLPAPIERTISKPKGSVRAPQVYVLPPPEEEMTKKQVTLTCMVTDFMPEDIYVEWTNNGKTELNYKNTEPVLDSDGSYFMYSKLRVEKKNWVERNSYSCSVVHEGLHNHHTTKSFSRTPGK

SEQ ID NO: 115 - protein, 184 aa, Artificial Sequence
  human BCMA (TNFRSF17) Protein NP_001183.2
MLQMAGQCSQNEYFDSLLHACIPCQLRCSSNTPPLTCQRYCNASVTNSVKGTNAILWTCLGLSLIISLAVFVLMFLLRKINSEPLKDEFKNTGSGLLGMANIDLEKSRTGDEIILPRGLEYTVEECTCEDCIKSKPKVDSDHCFPLPAMEEGATILVTTKTNDYCKSLPAALSATEIEKSISAR

SEQ ID NO: 116 - protein, 207 aa, Artificial Sequence
  human CD3 Epsilon Protein (>NP_000724.1 T-cell surface glycoprotein CD3 epsilon chain precursor
MQSGTHWRVLGLCLLSVGVWGQDGNEEMGGITQTPYKVSISGTTVILTCPQYPGSEILWQHNDKNIGGDEDDKNIGSDEDHLSLKEFSELEQSGYYVCYPRGSKPEDANFYLYLRARVCENCMEMDVMSVATIVIVDICITGGLLLLVYYWSKNRKAKAKPVTRGAGAGGRQRGQNKERPPPVPNPDYEPIRKGQRDLYSGLNQRRI

SEQ ID NO: 117 - protein, 171 aa, Artificial Sequence
  human CD3 Delta Protein (>NP_000723.1 T-cell surface glycoprotein CD3 delta chain isoform A precursor
MEHSTFLSGLVLATLLSQVSPFKIPIEELEDRVFVNCNTSITWVEGTVGTLLSDITRLDLGKRILDPRGIYRCNGTDIYKDKESTVQVHYRMCQSCVELDPATVAGIIVTDVIATLLLALGVFCFAGHETGRLSGAADTQALLRNDQVYQPLRDRDDAQYSHLGGNWARNK

SEQ ID NO: 118 - protein, 164 aa, Artificial Sequence
  human CD3 Zeta  Protein (>NP_932170.1 T-cell surface glycoprotein CD3 zeta chain isoform 1 precursor
MKWKALFTAAILQAQLPITEAQSFGLLDPKLCYLLDGILFIYGVILTALFLRVKFSRSADAPAYQQGQNQLYNELNLGRREEYDVLDKRRGRDPEMGGKPQRRKNPQEGLYNELQKDKMAEAYSEIGMKGERRRGKGHDGLYQGLSTATKDTYDALHMQALPPR

SEQ ID NO: 119 - protein, 182 aa, Artificial Sequence
  human CD3 Gamma Protein (>NP_000064.1 T-cell surface glycoprotein CD3 gamma chain precursor
MEQGKGLAVLILAIILLQGTLAQSIKGNHLVKVYDYQEDGSVLLTCDAEAKNITWFKDGKMIGFLTEDKKKWNLGSNAKDPRGMYQCKGSQNKSKPLQVYYRMCQNCIELNAATISGFLFAEIVSIFVLAVGVYFIAGQDGVRQSRASDKQTLLPNDQLYQPLKDREDDQYSHLQGNQLRRN

SEQ ID NO: 120 - protein, 281 aa, Artificial Sequence
  Human BCMA ecto.hFc Protein
MLQMAGQCSQNEYFDSLLHACIPCQLRCSSNTPPLTCQRYCNASVTNSVKGTNADKTHTCPPCPAPELLGGPSVFLFPPKPKDTLMISRTPEVTCVVVDVSHEDPEVKFNWYVDGVEVHNAKTKPREEQYNSTYRVVSVLTVLHQDWLNGKEYKCKVSNKALPAPIEKTISKAKGQPREPQVYTLPPSRDELTKNQVSLTCLVKGFYPSDIAVEWESNGQPENNYKTTPPVLDSDGSFFLYSKLTVDKSRWQQGNVFSCSVMHEALHNHYTQKSLSLSPGK

SEQ ID NO: 121 - protein, 43 aa, Artificial Sequence
  Peptides 1-43 of human BCMA
MLQMAGQCSQNEYFDSLLHACIPCQLRCSSNTPPLTCQRYCNA

SEQ ID NO: 122 - protein, 125 aa, Artificial Sequence
  21587N VH
QVQLQESGPGLVKPSETLSLTCTVSGGSINYYYWNWIRQPPGKGLEWIGYISYSGNTNYNPSLKSRVTISVATSRNQFSLTLSSVTAADTAVYYCARFAEYCGGNICYYYGMDVWGQGTTVTVSS

SEQ ID NO: 123 - protein, 108 aa, Artificial Sequence
  21587N VL (Non-germline Cys in CDR3)
EIVLTQSPGTLSLSPGERATFSCRASQSVGSSFLAWYQQKPGQAPRRLMYGASNRATGIPDRFSGSGSGTDFTLTISRLEPEDFAVYYCQQCGGSPWTFGQGTKVEIK

SEQ ID NO: 124 - protein, 127 aa, Artificial Sequence
  21589N VH
QVQLVQSGAEVKRPGSSVKVSCKASGGTFSTYAINWVRQAPGQGLEWMGGIIPIFGTTNYAQKFQGRVTITTDGSTTTTYMELSSLRSEDTAVYYCARTVYDLNSKGYYYYYGLDVWGQGTTVTVSS

SEQ ID NO: 125 - protein, 114 aa, Artificial Sequence
  21589N VL
DIVMTQTPLSLPVTPGEPASISCRSSQSLLDSDDGNTYLDWYLQKPGQSPQLLIYTLSYRASGVPDRFSGSGSGTDFTLKISRVEAEDVGIYYCMQRIEFPSLTFGGGTKVEIK